European Patent Specification EP 3 407 722 B1, published October 4, 2023. Title: MICROBIAL CONSORTIA. Applicant: Agrinos AS. The sequence listing filed with the application follows.

SEQUENCE LISTING (17 sequences)

SEQ ID NO: 1 - DNA, 1579 bp, Lactobacillus sp.
tatgagagtttgatcctggctcaggatgaacgctggcggcgtgcctaatacatgcaagtcgaacgagttctcgttgatgatcggtgcttgcaccgagattcaacatggaacgagtggcggacgggtgagtaacacgtgggtaacctgcccttaagtgggggataacatttggaaacagatgctaataccgcatagatccaagaaccgcatggttcttggctgaaagatggcgtaagctatcgcttttggatggacccgcggcgtattagctagttggtgaggtaacggctcaccaaggcgatgatacgtagccgaactgagaggttgatcggccacattgggactgagacacggcccaaactcctacgggaggcagcagtagggaatcttccacaatggacgcaagtctgatggagcaacgccgcgtgagtgaagaaggctttcgggtcgtaaaactctgttgttggagaagaatggtcggcagagtaactgttgtcggcgtgacggtatccaaccagaaagccacggctaactacgtgccagcagccgcggtaatacgtaggtggcaagcgttatccggatttattgggcgtaaagcgagcgcaggcggttttttaagtctgatgtgaaagccctcggcttaaccgaggaagcgcatcggaaactgggaaacttgagtgcagaagaggacagtggaactccatgtgtagcggtgaaatgcgtagatatatggaagaacaccagtggcgaaggcggctgtctggtctgtaactgacgctgaggctcgaaagcatgggtagcgaacaggattagataccctggtagtccatgccgtaaacgatgaatgctaggtgttggagggtttccgcccttcagtgccgcagctaacgcattaagcattccgcctggggagtacgaccgcaaggttgaaactcaaaggaattgacgggggcccgcacaagcggtggagcatgtggtttaattcgaagcaacgcgaagaaccttaccaggtcttgacatcttttgatcacctgagagatcaggtttccccttcgggggcaaaatgacaggtggtgcatggttgtcgtcagctcgtgtcgtgagatgttgggttaagtcccgcaacgagcgcaacccttatgactagttgccagcatttagttgggcactctagtaagactgccggtgacaaaccggaggaaggtggggatgacgtcaaatcatcatgccccttatgacctgggctacacacgtgctacaatggatggtacaacgagttgcgagaccgcgaggtcaagctaatctcttaaagccattctcagttcggactgtaggctgcaactcgcctacacgaagtcggaatcgctagtaatcgcggatcagcacgccgcggtgaatacgttcccgggccttgtacacaccgcccgtcacaccatgagagtttgtaacacccgaagccggtggcgtaacccttttagggagcgagccgtctaaggtgggacaaatgattagggtgaagtcgtaacaaggtagccgtaggagaacctgcggctggatcacctcctttaagcaccgatca

SEQ ID NO: 2 - DNA, 1510 bp, Clostridium beijerinckii
tattgagagtttgatcctggctcaggacgaacgctggcggcgtgcttaacacatgcaagtcgagcgatgaagttccttcgggaatggattagcggcggacgggtgagtaacacgtgggtaacctgcctcatagaggggaatagcctttcgaaaggaagattaataccgcataagattgtagtgccgcatggcatagcaattaaaggagtaatccgctatgagatggacccgcgtcgcattagctagttggtgaggtaacggctcaccaaggcgacgatgcgtagccgacctgagagggtgatcggccacattgggactgagacacggcccagactcctacgggaggcagcagtggggaatattgcacaatgggggaaaccctgatgcagcaacgccgcgtgagtgatgacggtcttcggattgtaaagctctgtcttcagggacgataatgacggtacctgaggaggaagccacggctaactacgtgccagcagccgcggtaatacgtaggtggcaagcgttgtccggatttactgggcgtaaagggagcgtaggtggatatttaagtgggatgtgaaatactcgggcttaacctgggtgctgcattccaaactggatatctagagtgcaggagaggaaagtagaattcctagtgtagcggtgaaatgcgtagagattaggaagaataccagtggcgaaggcgactttctggactgtaactgacactgaggctcgaaagcgtggggagcaaacaggattagataccctggtagtccacgccgtaaacgatgaatactaggtgtaggggttgtcatgacctctgtgccgccgctaacgcattaagtattccgcctggggagtacggtcgcaagattaaaactcaaaggaattgacgggggcccgcacaagcagcggagcatgtggtttaattcgaagcaacgcgaagaaccttacctagacttgacatctcctgaattacccttaatcggggaagcccttcggggcaggaagacaggtggtgcatggttgtcgtcagctcgtgtcgtgagatgttgggttaagtcccgcaacgagcgcaacccttattgttagttgctaccatttagttgagcactctagcgagactgcccgggttaaccgggaggaaggtggggatgacgtcaaatcatcatgccccttatgtctagggctacacacgtgctacaatggctggtacagagagatgctaaaccgtgaggtggagccaaactttaaaaccagtctcagttcggattgtaggctgaaactcgcctacatgaagctggagttgctagtaatcgcgaatcagaatgtcgcggtgaatacgttcccgggccttgtacacaccgcccgtcacaccatgagagttggcaatacccaaagttcgtgagctaacgcgcaagcggggcagcgacctaaggtagggtcagcgattggggtgaagtcgtaacaaggtagccgtaggagaacctgcggctggatcacctccttt

SEQ ID NO: 3 - DNA, 1485 bp, Acetobacter pasteurianus
cctgagagtttgatcctggctcagagcgaacgctggcggcatgcttaacacatgcaagtcgcacgaaggtttcggccttagtggcggacgggtgagtaacgcgtaggtatctatccatgggtgggggataacactgggaaactggtgctaataccgcatgacacctgagggtcaaaggcgcaagtcgcctgtggaggagcctgcgtttgattagctagttggtggggtaaaggcctaccaaggcgatgatcaatagctggtttgagaggatgatcagccacactgggactgagacacggcccagactcctacgggaggcagcagtggggaatattggacaatgggggcaaccctgatccagcaatgccgcgtgtgtgaagaaggtcttcggattgtaaagcactttcgacggggacgatgatgacggtacccgtagaagaagccccggctaacttcgtgccagcagccgcggtaatacgaagggggctagcgttgctcggaatgactgggcgtaaagggcgtgtaggcggtttgtacagtcagatgtgaaatccccgggcttaacctgggagctgcatttgatacgtgcagactagagtgtgagagagggttgtggaattcccagtgtagaggtgaaattcgtagatattgggaagaacaccggtggcgaaggcggcaacctggctcattactgacgctgaggcgcgaaagcgtggggagcaaacaggattagataccctggtagtccacgctgtaaacgatgtgtgctagatgttgggtgacttagtcattcagtgtcgcagttaacgcgttaagcacaccgcctggggagtacggccgcaaggttgaaactcaaaggaattgacgggggcccgcacaagcggtggagcatgtggtttaattcgaagcaacgcgcagaaccttaccagggcttgaatgtagaggctgcaagcagagatgtttgtttcccgcaagggacctctaacacaggtgctgcatggctgtcgtcagctcgtgtcgtgagatgttgggttaagtcccgcaacgagcgcaacccctatctttagttgccatcaggttgggctgggcactctagagagactgccggtgacaagccggaggaaggtggggatgacgtcaagtcctcatggcccttatgtcctgggctacacacgtgctacaatggcggtgacagtgggaagctaggtggtgacaccatgctgatctctaaaagccgtctcagttcggattgcactctgcaactcgagtgcatgaaggtggaatcgctagtaatcgcggatcagcatgccgcggtgaatacgttcccgggccttgtacacaccgcccgtcacaccatgggagttggtttgaccttaagccggtgagcgaaccgcaaggacgcagccgaccacggtcgggtcagcgactggggtgaagtcgtaacaaggtagccgtaggggaacctgcggctggatcacctccttt

SEQ ID NO: 4 - DNA, 1571 bp, Lactobacillus buchneri
atgagagtttgatcctggctcaggacgaacgctggcggcgtgcctaatacatgcaagtcgaacgcgtctccgttaatgattttaggtgcttgcacttgaaagatttaacattgagacgagtggcgaactggtgagtaacacgtgggtaacctgcccttgaagtaggggataacacttggaaacaggtgctaataccgtataacaaccaaaaccacctggttttggtttaaaagacggcttcggctgtcactttaggatggacccgcggcgtattagcttgttggtaaggtaacggcctaccaaggcgatgatacgtagccgacctgagagggtaatcggccacattgggactgagacacggcccaaactcctacgggaggcagcagtagggaatcttccacaatggacgaaagtctgatggagcaacgccgcgtgagtgatgaagggtttcggctcgtaaaactctgttgttggagaagaacaggtgtcagagtaactgttgacatcttgacggtatccaaccagaaagccacggctaactacgtgccagcagccgcggtaatacgtaggtggcaagcgttgtccggatttattgggcgtaaagcgagcgcaggcggttttttaggtctgatgtgaaagccttcggcttaaccggagaagtgcatcggaaaccgggagacttgagtgcagaagaggacagtggaactccatgtgtagcggtgaaatgcgtagatatatggaagaacaccagtggcgaaggcggctgtctggtctgtaactgacgctgaggctcgaaagcatgggtagcgaacaggattagataccctggtagtccatgccgtaaacgatgagtgctaagtgttggagggtttccgcccttcagtgctgcagctaacgcattaagcactccgcctggggagtacgaccgcaaggttgaaactcaaaggaattgacgggggcccgcacaagcggtggagcatgtggtttaattcgatgctacgcgaagaaccttaccaggtcttgacatcttctgccaacttaagagattaggcgttcccttcggggacagaatgacaggtggtgcatggttgtcgtcagctcgtgtcgtgagatgttgggttaagtcccgcaacgagcgcaacccttattgttagttgccagcattcagttgggcactctagcaagactgccggtgacaaaccggaggaaggtggggatgacgtcaaatcatcatgccccttatgacctgggctacacacgtgctacaatggacggtacaacgagtcgcgaaaccgcgaggtcaagctaatctcttaaagccgttctcagttcggattgtaggctgcaactcgcctacatgaagttggaatcgctagtaatcgtggatcagcatgccacggtgaatacgttcccgggccttgtacacaccgcccgtcacaccatgagagtttgtaacacccaaagccggtgaggtaaccttcggggaccagccgtctaaggtggggcagatgattagggtgaagtcgtaacaaggtagccgtaggagaacctgcggctggatcacctccttt

SEQ ID NO: 5 - DNA, 1548 bp, Bacillus subtilis
atcggagagtttgatcctggctcaggacgaacgctggcggcgtgcctaatacatgcaagtcgagcggacagatgggagcttgctccctgatgttagcggcggacgggtgagtaacacgtgggtaacctgcctgtaagactgggataactccgggaaaccggggctaataccggatggttgtttgaaccgcatggttcaaacataaaaggtggcttcggctaccacttacagatggacccgcggcgcattagctagttggtgaggtaacggctcaccaaggcaacgatgcgtagccgacctgagagggtgatcggccacactgggactgagacacggcccagactcctacgggaggcagcagtagggaatcttccgcaatggacgaaagtctgacggagcaacgccgcgtgagtgatgaaggttttcggatcgtaaagctctgttgttagggaagaacaagtaccgttcgaatagggcggtaccttgacggtacctaaccagaaagccacggctaactacgtgccagcagccgcggtaatacgtaggtggcaagcgttgtccggaattattgggcgtaaagggctcgcaggcggtttcttaagtctgatgtgaaagcccccggctcaaccggggagggtcattggaaactggggaacttgagtgcagaagaggagagtggaattccacgtgtagcggtgaaatgcgtagagatgtggaggaacaccagtggcgaaggcgactctctggtctgtaactgacgctgaggagcgaaagcgtggggagcgaacaggattagataccctggtagtccacgccgtaaacgatgagtgctaagtgttagggggtttccgccccttagtgctgcagctaacgcattaagcactccgcctggggagtacggtcgcaagactgaaactcaaaggaattgacgggggcccgcacaagcggtggagcatgtggtttaattcgaagcaacgcgaagaaccttaccaggtcttgacatcctctgacaatcctagagataggacgtccccttcgggggcagagtgacaggtggtgcatggttgtcgtcagctcgtgtcgtgagatgttgggttaagtcccgcaacgagcgcaacccttgatcttagttgccagcattcagttgggcactctaaggtgactgccggtgacaaaccggaggaaggtggggatgacgtcaaatcatcatgccccttatgacctgggctacacacgtgctacaatggacagaacaaagggcagcgaaaccgcgaggttaagccaatcccacaaatctgttctcagttcggatcgcagtctgcaactcgactgcgtgaagctggaatcgctagtaatcgcggatcagcatgccgcggtgaatacgttcccgggccttgtacacaccgcccgtcacaccacgagagtttgtaacacccgaagtcggtgaggtaaccttttaggagccagccgccgaaggtgggacagatgattggggtgaagtcgtaacaaggtagccgtatcggaaggtgcggctggatcacctccttt

SEQ ID NO: 6 - DNA, 1552 bp, Paenibacillus cookii
cttggagagtttgatcctggctcaggacgaacgctggcggcgtgcctaatacatgcaagtcgagcggagttgatggggagcttgctctcctgagacttagcggcggacgggtgagtaacacgtaggcaacctgcccgtaagaccgggataactaccggaaacggtagctaataccggataatttatcgcttcgcatggagcggtaatgaaagacggagcaatctgtcacttacggatgggcctgcggcgcattagctagttggtgaggtaacggctcaccaaggcgacgatgcgtagccgacctgagagggtgaacggccacactgggactgagacacggcccagactcctacgggaggcagcagtagggaatcttccgcaatgggcgaaagcctgacggagcaacgccgcgtgagtgatgaaggttttcggatcgtaaagctctgttgccagggaagaacgtcgggtagagtaactgctatccgagtgacggtacctgagaagaaagccccggctaactacgtgccagcagccgcggtaatacgtagggggcaagcgttgtccggaattattgggcgtaaagcgcgcgcaggcggtcacttaagtctggtgtttaaggctagggctcaactctagttcgcactggaaactgggtgacttgagtgcagaagaggaaagtggaattccacgtgtagcggtgaaatgcgtagagatgtggaggaacaccagtggcgaaggcgactttctgggctgtaactgacgctgaggcgcgaaagcgtggggagcaaacaggattagataccctggtagtccacgccgtaaacgatgaatgctaggtgttaggggtttcgatacccttggtgccgaagttaacacattaagcattccgcctggggagtacggtcgcaagactgaaactcaaaggaattgacggggacccgcacaagcagtggagtatgtggtttaattcgaagcaacgcgaagaaccttaccaggtcttgacatccctctgaatcctctagagatagaggcggccttcgggacagaggagacaggtggtgcatggttgtcgtcagctcgtgtcgtgagatgttgggttaagtcccgcaacgagcgcaacccttgattttagttgccagcacattaaggtgggcactctagaatgactgccggtgacaaaccggaggaaggcggggatgacgtcaaatcatcatgccccttatgacctgggctacacacgtactacaatggccagtacaacgggaagcgaagtcgcgagacggagccaatcctatcaaagctggtctcagttcggattgcaggctgcaacccgcctgcatgaagtcggaattgctagtaatcgcggatcagcatgccgcggtgaatacgttcccgggtcttgtacacaccgcccgtcacaccacgagagtttacaacacccgaagtcggtggggtaaccgcaaggagccagccgccgaaggtggggtagatgattggggtgaagtcgtaacaaggtagccgtatcggaaggtgcggctggatcacctccttt

SEQ ID NO: 7 - DNA, 1554 bp, Lactobacillus vini
aatgagagtttgatcctggctcaggacgaacgctggcggcgtgcctaatacatgcaagtcgaacgagactttttatttgatgcttgcatcttttaaaaagttgagtggcgaacgggtgagtaacacgtgggtaacctgccttaaagtgggggataacacttggaaacaggtgctaataccgcataaccatcaaaaccgcctggttttgatgttaaagatggttctgctatcgctttaagatggacccgcggcgtattagctagttggtgaggtaacggcttaccaaggcaatgatacgtagccgaactgagaggttgatcggccacattgggactgagacacggcccaaactcctacgggaggcagcagtagggaatctttcacaatggacgaaagtctgatggagcaacgccgcgtgagtgaagaaggttttcggatcgtaaaactctgttgtcagagaagaacgtgtgtgagagtaactgttcacgcagtgacggtatctgaccagaaagtcacggctaactacgtgccagcagccgcggtaatacgtaggtggcaagcgttgtccggatttattgggcgtaaagggaacgcaggcggtcttttaagtctgatgtgaaagccttcggcttaaccgaagtcgggcattggaaactgggagacttgagtgcagaagaggagagtggaactccatgtgtagcggtgaaatgcgtagatatatggaagaacaccagtggcgaaagcggctctctggtctgtaactgacgctgaggttcgaaagcgtgggtagcaaacaggattagataccctggtagtccacgccgtaaacgatgaatgctaagtgttggagggtttccgcccttcagtgccgcagctaacgcattaagcattccgcctggggagtacgatcgcaagattgaaactcaaaggaattgacgggggcccgcacaagcggtggagcatgtggtttaattcgaagcaacgcgaagaaccttaccaggtcttgacatcttttgctaacctgagagatcaggtgttcccttcggggacaaaatgacaggtggtgcatggttgtcgtcagctcgtgtcgtgagatgttgggttaagtcccgcaacgagcgcaacccttattgttagttgccagcatttagttgggcactctaacgagactgccggtgacaaaccggaggaaggtggggatgacgtcaaatcatcatgccccttatgacctgggctacacacgtgctacaatggacggtacaacgagtcgcaagaccgcgaggtcaagctaatctctgaaaaccgttctcagttcggattgcaggctgcaactcgcctgcatgaagtcggaatcgctagtaatcgcggatcagcatgccgcggtgaatacgttcccgggccttgtacacaccgcccgtcacaccatgagagtttgtaacacccaaagccggtggggtaacctttgggagccagccgtctaaggtgggacagatgattggggtgaagtcgtaacaaggtagccgtaggagaacctgcggctggatcacctccttt

SEQ ID NO: 8 - DNA, 1553 bp, Paenibacillus lautus
attggagagtttgatcctggctcaggacgaacgctggcggcgtgcctaatacatgcaagtcgagcggacttgatggagtgcttgcactcctgaaggttagcggcggacgggtgagtaacacgtaggcaacctgccctcaagactgggataactaccggaaacggtagctaataccggataatttattttgcagcattgtgaaataatgaaaggcggagcaatctgtcacttgaggatgggcctgcggcgcattagctagttggtggggtaacggcccaccaaggcgacgatgcgtagccgacctgagagggtgaacggccacactgggactgagacacggcccagactcctacgggaggcagcagtagggaatcttccgcaatgggcgaaagcctgacggagcaacgccgcgtgagtgatgaaggttttcggatcgtaaagctctgttgccaaggaagaacgtcttctagagtaactgctaggagagtgacggtacttgagaagaaagccccggctaactacgtgccagcagccgcggtaatacgtagggggcaagcgttgtccggaattattgggcgtaaagcgcgcgcaggcggttctttaagtctggtgtttaaacccgaggctcaacttcgggtcgcactggaaactggggaacttgagtgcagaagaggagagtggaattccacgtgtagcggtgaaatgcgtagatatgtggaggaacaccagtggcgaaggcgactctctgggctgtaactgacgctgaggcgcgaaagcgtggggagcaaacaggattagataccctggtagtccacgccgtaaacgatgaatgctaggtgttaggggtttcgatacccttggtgccgaagttaacacattaagcattccgcctggggagtacggtcgcaagactgaaactcaaaggaattgacggggacccgcacaagcagtggagtatgtggtttaattcgaagcaacgcgaagaaccttaccaagtcttgacatccctctgaatcctctagagatagaggcggccttcgggacagaggtgacaggtggtgcatggttgtcgtcagctcgtgtcgtgagatgttgggttaagtcccgcaacgagcgcaacccttgattttagttgccagcacttcgggtgggcactctagaatgactgccggtgacaaaccggaggaaggcggggatgacgtcaaatcatcatgccccttatgacttgggctacacacgtactacaatggctggtacaacgggaagcgaagccgcgaggtggagccaatcctataaaagccagtctcagttcggattgcaggctgcaactcgcctgcatgaagtcggaattgctagtaatcgcggatcagcatgccgcggtgaatacgttcccgggtcttgtacacaccgcccgtcacaccacgagagtttacaacacccgaagtcggtggggtaacccttaggggagccagccgccgaaggtggggtagatgattggggtgaagtcgtaacaaggtagccgtatcggaaggtgcggctggatcacctccttt

SEQ ID NO: 9 - DNA, 1561 bp, Oceanobacillus oncorhynchi subsp. incaldanensis
ttatggagagtttgatcttggctcaggacgaacgctggcggcgtgcctaatacatgcaagtcgagcgcgggaagcgaacggaactcttcggagggaagttcgtggaacgagcggcggacgggtgagtaacacgtaggcaacctgcctgtaagactgggataactcgcggaaacgcgagctaataccggataacactttctatcacctgatggaaagttgaaaggcggcttttgctgtcacttacagatgggcctgcggcgcattagctagttggtgaggtaacggctcaccaaggcgacgatgcgtagccgacctgagagggtgatcggccacactgggactgagacacggcccagactcctacgggaggcagcagtagggaatcttccgcaatggacgaaagtctgacggagcaacgccgcgtgagtgatgaaggttttcggatcgtaaaactctgttgtcagggaagaacaagtacgatagtaactgatcgtaccttgacggtacctgaccagaaagccacggctaactacgtgccagcagccgcggtaatacgtaggtggcaagcgttgtccggaattattgggcgtaaagcgctcgcaggcggttctttaagtctgatgtgaaatcttgcggctcaaccgcaaacgtgcattggaaactggaggacttgagtgcagaagaggagagtggaattccacgtgtagcggtgaaatgcgtagagatgtggaggaacaccagtggcgaaggcgactctctggtctgtaactgacgctgaggagcgaaagcgtggggagcgaacaggattagataccctggtagtccacgccgtaaacgatgagtgctaggtgttagggggtttccgccccttagtgctgaagttaacgcattaagcactccgcctggggagtacggccgcaaggctgaaactcaaaagaattgacggggacccgcacaagcggtggagcatgtggtttaattcgaagcaacgcgaagaaccttaccaggtcttgacatcctttgaccgctctagagatagagttttcccttcggggacaaagtgacaggtggtgcatggttgtcgtcagctcgtgtcgtgagatgttgggttaagtcccgcaacgagcgcaacccttaatcttagttgccagcatttagttgggcactctaaggtgactgccggtgacaaaccggaggaaggtggggatgacgtcaaatcatcatgccccttatgacctgggctacacacgtgctacaatggacggaacaaagggaagcgaacccgcgaggtccagcaaatcccataaaaccgttctcagttcggattgcaggctgcaactcgcctgcatgaagccggaatcgctagtaatcgcggatcagcatgccgcggtgaatacgttcccgggtcttgtacacaccgcccgtcacaccacgagagttcgtaacacccgaagtcggtgaggtaaccttttggagccagccgccgaaggtgggacgaatgattggggtgaagtcgtaacaaggtagccgtatcggaaggtgcggctggatcacctccttt

SEQ ID NO: 10 - DNA, 1548 bp, Bacillus amyloliquefaciens
atcggagagtttgatcctggctcaggacgaacgctggcggcgtgcctaatacatgcaagtcgagcggacagatgggagcttgctccctgatgttagcggcggacgggtgagtaacacgtgggtaacctgcctgtaagactgggataactccgggaaaccggggctaataccggatggttgtctgaaccgcatggttcagacataaaaggtggcttcggctaccacttacagatggacccgcggcgcattagctagttggtgaggtaacggctcaccaaggcgacgatgcgtagccgacctgagagggtgatcggccacactgggactgagacacggcccagactcctacgggaggcagcagtagggaatcttccgcaatggacgaaagtctgacggagcaacgccgcgtgagtgatgaaggttttcggatcgtaaagctctgttgttagggaagaacaagtgccgttcaaatagggcggcaccttgacggtacctaaccagaaagccacggctaactacgtgccagcagccgcggtaatacgtaggtggcaagcgttgtccggaattattgggcgtaaagggctcgcaggcggtttcttaagtctgatgtgaaagcccccggctcaaccggggagggtcattggaaactggggaacttgagtgcagaagaggagagtggaattccacgtgtagcggtgaaatgcgtagagatgtggaggaacaccagtggcgaaggcgactctctggtctgtaactgacgctgaggagcgaaagcgtggggagcgaacaggattagataccctggtagtccacgccgtaaacgatgagtgctaagtgttagggggtttccgccccttagtgctgcagctaacgcattaagcactccgcctggggagtacggtcgcaagactgaaactcaaaggaattgacgggggcccgcacaagcggtggagcatgtggtttaattcgaagcaacgcgaagaaccttaccaggtcttgacatcctctgacaatcctagagataggacgtccccttcgggggcagagtgacaggtggtgcatggttgtcgtcagctcgtgtcgtgagatgttgggttaagtcccgcaacgagcgcaacccttgatcttagttgccagcattcagttgggcactctaaggtgactgccggtgacaaaccggaggaaggtggggatgacgtcaaatcatcatgccccttatgacctgggctacacacgtgctacaatggacagaacaaagggcagcgaaaccgcgaggttaagccaatcccacaaatctgttctcagttcggatcgcagtctgcaactcgactgcgtgaagctggaatcgctagtaatcgcggatcagcatgccgcggtgaatacgttcccgggccttgtacacaccgcccgtcacaccacgagagtttgtaacacccgaagtcggtgaggtaacctttatggagccagccgccgaaggtgggacagatgattggggtgaagtcgtaacaaggtagccgtatcggaaggtgcggctggatcacctccttt

SEQ ID NO: 11 - DNA, 1547 bp, Bacillus sp.
attggagagtttgatcctggctcaggacgaacgctggcggcgtgcctaatacatgcaagtcgagcgaatctgagggagcttgctcccaaagattagcggcggacgggtgagtaacacgtgggcaacctgcctgtaagactgggataactccgggaaaccggggctaataccggataatatctatttatacatataattagattgaaagatggttctgctatcacttacagatgggcccgcggcgcattagctagttggtgaggtaacggctcaccaaggcgacgatgcgtagccgacctgagagggtgatcggccacactgggactgagacacggcccagactcctacgggaggcagcagtagggaatcttccgcaatggacgaaagtctgacggagcaacgccgcgtgagtgatgaaggttttcggatcgtaaaactctgttgttagggaagaacaagtatcggagtaactgccggtaccttgacggtacctaaccagaaagccacggctaactacgtgccagcagccgcggtaatacgtaggtggcaagcgttgtccggaattattgggcgtaaagcgcgcgcaggcggttccttaagtctgatgtgaaagcccacggctcaaccgtggagggtcattggaaactggggaacttgagtgcagaagaggaaagtggaattccaagtgtagcggtgaaatgcgtagagatttggaggaacaccagtggcgaaggcgactttctggtctgtaactgacgctgaggcgcgaaagcgtggggagcaaacaggattagataccctggtagtccacgccgtaaacgatgagtgctaagtgttagagggtttccgccctttagtgctgcagcaaacgcattaagcactccgcctggggagtacgaccgcaaggttgaaactcaaaggaattgacgggggcccgcacaagcggtggagcatgtggtttaattcgaagcaacgcgaagaaccttaccaggtcttgacatcctctgacaatcctagagataggactttccccttcgggggacagagtgacaggtggtgcatggttgtcgtcagctcgtgtcgtgagatgttgggttaagtcccgcaacgagcgcaacccttgatcttagttgccagcatttagttgggcactctaaggtgactgccggtgacaaaccggaggaaggtggggatgacgtcaaatcatcatgccccttatgacctgggctacacacgtgctacaatggatggtacaaagggctgcaagaccgcgaggtttagccaatcccataaaaccattctcagttcggattgtaggctgcaactcgcctacatgaagccggaatcgctagtaatcgcggatcagcatgccgcggtgaatacgttcccgggccttgtacacaccgcccgtcacaccacgagagtttgtaacacccgaagtcggtggggtaaccttttggagccagccgcctaaggtgggacagatgattggggtgaagtcgtaacaaggtagccgtatcggaaggtgcggctggatcacctccttt

SEQ ID NO: 12 - DNA, 1553 bp, Paenibacillus chibensis
cttggagagtttgatcctggctcaggacgaacgctggcggcgtgcctaatacatgcaagtcgagcggagttgatgaggtgcttgcacctctgatgcttagcggcggacgggtgagtaacacgtaggtaacctgcctgtaagactgggataactaccggaaacggtagctaataccggataatttattttctctcctggggagataatgaaagacggagcaatctgtcacttacagatgggcctgcggcgcattagctagttggtgaggtaacggctcaccaaggcgacgatgcgtagccgacctgagagggtgaacggccacactgggactgagacacggcccagactcctacgggaggcagcagtagggaatcttccgcaatggacgaaagtctgacggagcaacgccgcgtgagtgatgaaggttttcggatcgtaaagctctgttgccagggaagaacgtccggtagagtaactgctaccggagtgacggtacctgagaagaaagccccggctaactacgtgccagcagccgcggtaatacgtagggggcaagcgttgtccggaattattgggcgtaaagcgcgcgcaggcggtcacttaagtctggtgtttaaggccaaggctcaaccttggttcgcactggaaactgggtgacttgagtgcagaagaggagagtggaattccacgtgtagcggtgaaatgcgtagatatgtggaggaacaccagtggcgaaggcgactctctgggctgtaactgacgctgaggcgcgaaagcgtggggagcaaacaggattagataccctggtagtccacgccgtaaacgatgaatgctaggtgttaggggtttcgatacccttggtgccgaagttaacacattaagcattccgcctggggagtacggtcgcaagactgaaactcaaaggaattgacggggacccgcacaagcagtggagtatgtggtttaattcgaagcaacgcgaagaaccttaccaagtcttgacatccctctgaatcctctagagatagaggcggccttcgggacagaggtgacaggtggtgcatggttgtcgtcagctcgtgtcgtgagatgttgggttaagtcccgcaacgagcgcaacccttgattttagttgccagcatttcggatgggcactctagaatgactgccggtgacaaaccggaggaaggcggggatgacgtcaaatcatcatgccccttatgacttgggctacacacgtactacaatggccagtacaacgggaagcgaaatcgcgagatggagccaatcctatcaaagctggtctcagttcggattgcaggctgcaacccgcctgcatgaagtcggaattgctagtaatcgcggatcagcatgccgcggtgaatacgttcccgggtcttgtacacaccgcccgtcacaccacgagagtttacaacacccgaagtcggtggggtaacccgcaagggagccagccgccgaaggtggggtagatgattggggtgaagtcgtaacaaggtagccgtatcggaaggtgcggctggatcacctccttt

SEQ ID NO: 13 - DNA, 1550 bp, Bacillus flexus
tcggagagtttgatcctggctcaggatgaacgctggcggcgtgcctaatacatgcaagtcgagcgaactgattagaagcttgcttctatgacgttagcggcggacgggtgagtaacacgtgggcaacctgcctgtaagactgggataactccgggaaaccggagctaataccggataacattttctcttgcataagagaaaattgaaagatggtttcggctatcacttacagatgggcccgcggtgcattagctagttggtgaggtaacggctcaccaaggcaacgatgcatagccgacctgagagggtgatcggccacactgggactgagacacggcccagactcctacgggaggcagcagtagggaatcttccgcaatggacgaaagtctgacggagcaacgccgcgtgagtgatgaaggctttcgggtcgtaaaactctgttgttagggaagaacaagtacaagagtaactgcttgtaccttgacggtacctaaccagaaagccacggctaactacgtgccagcagccgcggtaatacgtaggtggcaagcgttatccggaattattgggcgtaaagcgcgcgcaggcggtttcttaagtctgatgtgaaagcccacggctcaaccgtggagggtcattggaaactggggaacttgagtgcagaagagaaaagcggaattccacgtgtagcggtgaaatgcgtagagatgtggaggaacaccagtggcgaaggcggctttttggtctgtaactgacgctgaggcgcgaaagcgtggggagcaaacaggattagataccctggtagtccacgccgtaaacgatgagtgctaagtgttagagggtttccgccctttagtgctgcagctaacgcattaagcactccgcctggggagtacggtcgcaagactgaaactcaaaggaattgacgggggcccgcacaagcggtggagcatgtggtttaattcgaagcaacgcgaagaaccttaccaggtcttgacatcctctgacaactctagagatagagcgttccccttcgggggacagagtgacaggtggtgcatggttgtcgtcagctcgtgtcgtgagatgttgggttaagtcccgcaacgagcgcaacccttgatcttagttgccagcatttagttgggcactctaaggtgactgccggtgacaaaccggaggaaggtggggatgacgtcaaatcatcatgccccttatgacctgggctacacacgtgctacaatggatggtacaaagggctgcaagaccgcgaggtcaagccaatcccataaaaccattctcagttcggattgtaggctgcaactcgcctacatgaagctggaatcgctagtaatcgcggatcagcatgccgcggtgaatacgttcccgggccttgtacacaccgcccgtcacaccacgagagtttgtaacacccgaagtcggtggggtaacctttatggagccagccgcctaaggtgggacagatgattggggtgaagtcgtaacaaggtagccgtatcggaaggtgcggctggatcacctccttt

SEQ ID NO: 14 - DNA, 1505 bp, Clostridium pasteurianum
aattgagagtttgatcctggctcaggacgaacgctggcggcgtgcttaacacatgcaagtcgagcgagaaaccttcgggtttctagcggcggacgggtgagtaacacgtgggtaacctgcctcaaagaggggaatagcctcccgaaagggagattaataccgcataatattacagcttcgcatgaagcagtaattaaaggagtaatccgctttgagatggacccgcggcgcattagctagttggagaggtaacggctcaccaaggcgacgatgcgtagccgacctgagagggtgatcggccacattggaactgagacacggtccagactcctacgggaggcagcagtggggaatattgcacaatgggcgaaagcctgatgcagcaacgccgcgtgagtgatgacggtcttcggattgtaaagctctgtcttttgggacgataatgacggtaccaaaggaggaagccacggctaactacgtgccagcagccgcggtaatacgtaggtggcaagcgttgtccggatttactgggcgtaaaggatgtgtaggcggatacttaagtgagatgtgaaagccccgggcttaacttggggactgcatttcaaactgggtgtctagagtgcaggagaggaaagcggaattcctagtgtagcggtgaaatgcgtagagattaggaagaacatcagtggcgaaggcggctttctggactgtaactgacgctgaggcatgaaagcgtggggagcaaacaggattagataccctggtagtccacgccgtaaacgatgagtactaggtgtaggaggtatcgactccttctgtgccgcagtaaacacaataagtactccgcctgggaagtacggtcgcaagattaaaactcaaaggaattgacgggggcccgcacaagcagcggagcatgtggtttaattcgaagcaacgcgaagaaccttacctagacttgacatctcctgaatagcgtagagatacgtgaagcccttcggggcaggaagacaggtggtgcatggttgtcgtcagctcgtgtcgtgagatgttgggttaagtcccgcaacgagcgcaacccttatcattagttgctaccattaagttgagcactctagtgagactgcccgggttaaccgggaggaaggcggggatgacgtcaaatcatcatgccccttatgtctagggctacacacgtgctacaatggtgagaacaacgagatgcaataccgcgaggtggagccaaacttgaaaactcatcccagttcggattgtaggctgaaattcgcctacatgaagttggagttgctagtaatcgcgaatcagaatgtcgcggtgaatacgttcccgggccttgtacacaccgcccgtcacaccatgagagctggtaacacccgaagtccgtgaggtaacctttatggagccagcggccgaaggtgggattagtgattggggtgaagtcgtaacaaggtagccgtaggagaacctgcggctggatcacctccttt

SEQ ID NO: 15 - DNA, 1566 bp, Virgibacillus halophilus
ttttggagagtttgatcttggctcaggacgaacgctggcggcgtgcctaatacatgcaagtcgagcgcgggaagcaggatgatcctcatctgaggtgattcctgtggaacgagcggcggacgggtgagtaacacgtgggcaacctgcctgtaagatcgggataactcgtggaaacgcgagctaataccggatgatacttttcatcgcatggtgagaagttgaaagatggctttaagctatcacttacagatgggcccgcggcgcattagctagttggtggggtaacggcctaccaaggcaacgatgcgtagccgacctgagagggtgatcggccacactgggactgagacacggcccagactcctacgggaggcagcagtagggaatcttccgcaatggacgaaagtctgacggagcaacgccgcgtgagtgatgaaggttttcggatcgtaaaactctgttgtcagggaagaacaagtgccgtttgaataaggcggcaccttgacggtacctgaccagaaagccccggctaactacgtgccagcagccgcggtaatacgtagggggcaagcgttgtccggaattattgggcgtaaagcgcgcgcaggcggtcttttaagtctgatgtgaaagcccacggcttaaccgtggagggtcattggaaactggaggacttgagtgcagaagaggagagtggaattccatgtgtagcggtgaaatgcgtagagatatggaggaacaccagtggcgaaggcgactctctggtctgcaactgacgctgaggcgcgaaagcgtgggtagcgaacaggattagataccctggtagtccacgccgtaaacgatgagtgctaggtgttagggggtttccgccccttagtgctgaagttaacgcattaagcactccgcctggggagtacggccgcaaggctgaaactcaaaagaattgacgggggcccgcacaagcggtggagcatgtggtttaattcgaagcaacgcgaagaaccttaccaggtcttgacatcctctgacagccttagagataaggtgttcccttcggggacagagtgacaggtggtgcatggttgtcgtcagctcgtgtcgtgagatgttgggttaagtcccgcaacgagcgcaacccttgagattagttgccagcattaagttgggcactctaatctgactgccggtgacaaaccggaggaaggtggggatgacgtcaaatcatcatgccccttatgacctgggctacacacgtgctacaatggatggtacagagggaagcgaagccgcgaggtgaagcaaatcccacaaaaccattctcagttcggattgcaggctgcaactcgcctgcatgaagccggaatcgctagtaatcgcggatcagcatgccgcggtgaatacgttcccgggccttgtacacaccgcccgtcacaccacgagagttggtaacacccgaagtcggtgaggtaacctttttggagccagccgccgaaggtgggacgaatgattggggtgaagtcgtaacaaggtagccgtatcggaaggtgcggctggatcacctccttt

SEQ ID NO: 16 - DNA, 1549 bp, Bacillus licheniformis
catggagagtttgatcctggctcaggacgaacgctggcggcgtgcctaatacatgcaagtcgagcggaccgacgggagcttgctcccttaggtcagcggcggacgggtgagtaacacgtgggtaacctgcctgtaagactgggataactccgggaaaccggggctaataccggatgcttgattgaaccgcatggttccaatcataaaaggtggcttttagctaccacttacagatggacccgcggcgcattagctagttggtgaggtaacggctcaccaaggcgacgatgcgtagccgacctgagagggtgatcggccacactgggactgagacacggcccagactcctacgggaggcagcagtagggaatcttccgcaatggacgaaagtctgacggagcaacgccgcgtgagtgatgaaggttttcggatcgtaaaactctgttgttagggaagaacaagtaccgttcgaatagggcggcaccttgacggtacctaaccagaaagccacggctaactacgtgccagcagccgcggtaatacgtaggtggcaagcgttgtccggaattattgggcgtaaagcgcgcgcaggcggtttcttaagtctgatgtgaaagcccccggctcaaccggggagggtcattggaaactggggaacttgagtgcagaagaggagagtggaattccacgtgtagcggtgaaatgcgtagagatgtggaggaacaccagtggcgaaggcgactctctggtctgtaactgacgctgaggcgcgaaagcgtggggagcgaacaggattagataccctggtagtccacgccgtaaacgatgagtgctaagtgttagagggtttccgccctttagtgctgcagcaaacgcattaagcactccgcctggggagtacggtcgcaagactgaaactcaaaggaattgacgggggcccgcacaagcggtggagcatgtggtttaattcgaagcaacgcgaagaaccttaccaggtcttgacatcctctgacaaccctagagatagggcttccccttcgggggcagagtgacaggtggtgcatggttgtcgtcagctcgtgtcgtgagatgttgggttaagtcccgcaacgagcgcaacccttgatcttagttgccagcattcagttgggcactctaaggtgactgccggtgacaaaccggaggaaggtggggatgacgtcaaatcatcatgccccttatgacctgggctacacacgtgctacaatgggcagaacaaagggcagcgaagccgcgaggctaagccaatcccacaaatctgttctcagttcggatcgcagtctgcaactcgactgcgtgaagctggaatcgctagtaatcgcggatcagcatgccgcggtgaatacgttcccgggccttgtacacaccgcccgtcacaccacgagagtttgtaacacccgaagtcggtgaggtaaccttttggagccagccgccgaaggtgggacagatgattggggtgaagtcgtaacaaggtagccgtatcggaaggtgcggctggatcacctccttt

SEQ ID NO: 17 - DNA, 1523 bp, Streptomyces griseus
acggagagtttgatcctggctcaggacgaacgctggcggcgtgcttaacacatgcaagtcgaacgatgaagcctttcggggtggattagtggcgaacgggtgagtaacacgtgggcaatctgcccttcactctgggacaagccctggaaacggggtctaataccggataacactctgtcccgcatgggacggggttaaaagctccggcggtgaaggatgagcccgcggcctatcagcttgttggtggggtaatggcctaccaaggcgacgacgggtagccggcctgagagggcgaccggccacactgggactgagacacggcccagactcctacgggaggcagcagtggggaatattgcacaatgggcgaaagcctgatgcagcgacgccgcgtgagggatgacggccttcgggttgtaaacctctttcagcagggaagaagcgagagtgacggtacctgcagaagaagcgccggctaactacgtgccagcagccgcggtaatacgtagggcgcaagcgttgtccggaattattgggcgtaaagagctcgtaggcggcttgtcacgtcggatgtgaaagcccggggcttaaccccgggtctgcattcgatacgggctagctagagtgtggtaggggagatcggaattcctggtgtagcggtgaaatgcgcagatatcaggaggaacaccggtggcgaaggcggatctctgggccattactgacgctgaggagcgaaagcgtggggagcgaacaggattagataccctggtagtccacgccgtaaacgttgggaactaggtgttggcgacattccacgtcgtcggtgccgcagctaacgcattaagttccccgcctggggagtacggccgcaaggctaaaactcaaaggaattgacgggggcccgcacaagcagcggagcatgtggcttaattcgacgcaacgcgaagaaccttaccaaggcttgacatataccggaaagcatcagagatggtgccccccttgtggtcggtatacaggtggtgcatggctgtcgtcagctcgtgtcgtgagatgttgggttaagtcccgcaacgagcgcaacccttgttctgtgttgccagcatgcccttcggggtgatggggactcacaggagactgccggggtcaactcggaggaaggtggggacgacgtcaagtcatcatgccccttatgtcttgggctgcacacgtgctacaatggccggtacaatgagctgcgatgccgcgaggcggagcgaatctcaaaaagccggtctcagttcggattggggtctgcaactcgaccccatgaagtcggagttgctagtaatcgcagatcagcattgctgcggtgaatacgttcccgggccttgtacacaccgcccgtcacgtcacgaaagtcggtaacacccgaagccggtggcccaaccccttgtgggagggagctgtcgaaggtgggactggcgattgggacgaagtcgtaacaaggtagccgtaccggaaggtgcggctggatcacctccttt